European Patent Application EP 4 707 390 A1, published March 11, 2026. Title: linker. Applicant: PeptiDream Inc. The sequence listing filed with the application follows.

SEQUENCE LISTING (60 sequences)

SEQ ID NO: 1 - DNA, 21 bp, synthetic construct
  source 1..21: mol_type = other DNA
cccgcctcccgccccccgtcc

SEQ ID NO: 2 - DNA, 90 bp, synthetic construct
  source 1..90: mol_type = other DNA
taagaaggagatatacatatgcgttgtgttaattttagtgatggttctactcctgctcttcatatttattggggaggtggtggaagtagc

SEQ ID NO: 3 - DNA, 60 bp, synthetic construct
  source 1..60: mol_type = other DNA
taagaaggagatatacatatgagtcatcctcaatttgaaaaaggaggtggtggaagtagt

SEQ ID NO: 4 - DNA, 87 bp, synthetic construct
  source 1..87: mol_type = other DNA
taagaaggagatatacatatgcgcttctgcaccggccacttcggcggcctctacccctgcaacggccccggaggtggtggaagtagt

SEQ ID NO: 5 - DNA, 90 bp, synthetic construct
  source 1..90: mol_type = other DNA
taagaaggagatatacatatgtggcacaagaacaagtacgtcctcacctactcctgcctcttcgccgccggcggaggtggtggaagtagc

SEQ ID NO: 6 - DNA, 81 bp, synthetic construct
  source 1..81: mol_type = other DNA
taagaaggagatatacatatgcccgactgcgcctaccacaagggcgagctcgtctggtgcaccggaggtggtggaagtagc

SEQ ID NO: 7 - DNA, 52 bp, synthetic construct
  source 1..52: mol_type = other DNA
ctagtaatacgactcactatagggttaactttaagaaggagatatacatatg

SEQ ID NO: 8 - DNA, 44 bp, synthetic construct
  source 1..44: mol_type = other DNA
cccgcctcccgccccccgtcctagctacttccaccacctcccca

SEQ ID NO: 9 - DNA, 23 bp, synthetic construct
  source 1..23: mol_type = other DNA
tagctacttccaccacctcccca

SEQ ID NO: 10 - DNA, 47 bp, synthetic construct
  source 1..47: mol_type = other DNA
cccgcctcccgccccccgtcctaactacttccaccacctcctttttc

SEQ ID NO: 11 - DNA, 44 bp, synthetic construct
  source 1..44: mol_type = other DNA
cccgcctcccgccccccgtcctaactacttccaccacctccggg

SEQ ID NO: 12 - DNA, 44 bp, synthetic construct
  source 1..44: mol_type = other DNA
cccgcctcccgccccccgtcctagctacttccaccacctccgcc

SEQ ID NO: 13 - DNA, 44 bp, synthetic construct
  source 1..44: mol_type = other DNA
cccgcctcccgccccccgtcctagctacttccaccacctccggt

SEQ ID NO: 14 - DNA, 23 bp, synthetic construct
  source 1..23: mol_type = other DNA
taactacttccaccacctccttt

SEQ ID NO: 15 - DNA, 23 bp, synthetic construct
  source 1..23: mol_type = other DNA
taactacttccaccacctccggg

SEQ ID NO: 16 - DNA, 23 bp, synthetic construct
  source 1..23: mol_type = other DNA
tagctacttccaccacctccgcc

SEQ ID NO: 17 - DNA, 23 bp, synthetic construct
  source 1..23: mol_type = other DNA
tagctacttccaccacctccggt

SEQ ID NO: 18 - DNA, 144 bp, synthetic construct
  source 1..144: mol_type = other DNA
ctagtaatacgactcactatagggttaactttaagaaggagatatacatatgcgttgtgttaattttagtgatggttctactcctgctcttcatatttattggggaggtggtggaagtagctaggacggggggcgggaggcggg

SEQ ID NO: 19 - protein, 24 aa, synthetic construct
  MUTAGEN 1: note = X stands for N-(3',6'-dihydroxy-3-oxo-3H-spiro[isobenzofuran-1,9'-xanthene]-5-carbonyl)-L-phenylalaninate
  MUTAGEN 3: note = X stand for N-methyl-L-alanine
XRXVNFSDGSTPALHIYWGGGGSS

SEQ ID NO: 20 - DNA, 114 bp, synthetic construct
  source 1..114: mol_type = other DNA
ctagtaatacgactcactatagggttaactttaagaaggagatatacatatgagtcatcctcaatttgaaaaaggaggtggtggaagtagttaggacggggggcgggaggcggg

SEQ ID NO: 21 - protein, 14 aa, synthetic construct
WSHPQFEKGGGGSS

SEQ ID NO: 22 - DNA, 141 bp, synthetic construct
  source 1..141: mol_type = other DNA
ctagtaatacgactcactatagggttaactttaagaaggagatatacatatgcgcttctgcaccggccacttcggcggcctctacccctgcaacggccccggaggtggtggaagtagttaggacggggggcgggaggcggg

SEQ ID NO: 23 - protein, 23 aa, synthetic construct
MRFCTGHFGGLYPCNGPGGGGSS

SEQ ID NO: 24 - DNA, 144 bp, synthetic construct
  source 1..144: mol_type = other DNA
ctagtaatacgactcactatagggttaactttaagaaggagatatacatatgtggcacaagaacaagtacgtcctcacctactcctgcctcttcgccgccggcggaggtggtggaagtagctaggacggggggcgggaggcggg

SEQ ID NO: 25 - protein, 24 aa, synthetic construct
  MUTAGEN 1: note = X stands for N-(2-chloroacetyl)-L-tyrosine
XWHKNKYVLTYSCLFAAGGGGGSS

SEQ ID NO: 26 - DNA, 135 bp, synthetic construct
  source 1..135: mol_type = other DNA
ctagtaatacgactcactatagggttaactttaagaaggagatatacatatgcccgactgcgcctaccacaagggcgagctcgtctggtgcaccggaggtggtggaagtagctaggacggggggcgggaggcggg

SEQ ID NO: 27 - protein, 21 aa, synthetic construct
MPDCAYHKGELVWCTGGGGSS

SEQ ID NO: 28 - RNA, 46 nt, synthetic construct
  source 1..46: mol_type = other RNA
ggatcgaaagatttccgcatccccgaaagggtacatggcgttaggt

SEQ ID NO: 29 - RNA, 45 nt, synthetic construct
  source 1..45: mol_type = other RNA
ggatcgaaagatttccgcggccccgaaaggggattagcgttaggt

SEQ ID NO: 30 - RNA, 77 nt, synthetic construct
  source 1..77: mol_type = other RNA
ggcggggtggagcagcctggtagctcgtcgggctcataacccgaagatcgtcggttcaaatccggcccccgcaacca

SEQ ID NO: 31 - RNA, 77 nt, synthetic construct
  source 1..77: mol_type = other RNA
gggtgattggcgcagcctggtagcgcacttcgctgcaaacgaaggggtcaggggttcgaatcccctatcacccgcca

SEQ ID NO: 32 - DNA, 54 bp, synthetic construct
  source 1..54: mol_type = other DNA
taagaaggagatatacatatgnntnntnntnnttggggaggtggtggaagtagc

SEQ ID NO: 33 - DNA, 57 bp, synthetic construct
  source 1..57: mol_type = other DNA
taagaaggagatatacatatgnntnntnntnntnnttggggaggtggtggaagtagc

SEQ ID NO: 34 - DNA, 60 bp, synthetic construct
  source 1..60: mol_type = other DNA
taagaaggagatatacatatgnntnntnntnntnntnnttggggaggtggtggaagtagc

SEQ ID NO: 35 - DNA, 63 bp, synthetic construct
  source 1..63: mol_type = other DNA
taagaaggagatatacatatgnntnntnntnntnntnntnnttggggaggtggtggaagtagc

SEQ ID NO: 36 - DNA, 66 bp, synthetic construct
  source 1..66: mol_type = other DNA
taagaaggagatatacatatgnntnntnntnntnntnntnntnnttggggaggtggtggaagtagc

SEQ ID NO: 37 - DNA, 69 bp, synthetic construct
  source 1..69: mol_type = other DNA
taagaaggagatatacatatgnntnntnntnntnntnntnntnntnnttggggaggtggtggaagtagc

SEQ ID NO: 38 - DNA, 72 bp, synthetic construct
  source 1..72: mol_type = other DNA
taagaaggagatatacatatgnntnntnntnntnntnntnntnntnntnnttggggaggtggtggaagtagc

SEQ ID NO: 39 - DNA, 75 bp, synthetic construct
  source 1..75: mol_type = other DNA
taagaaggagatatacatatgnntnntnntnntnntnntnntnntnntnntnnttggggaggtggtggaagtagc

SEQ ID NO: 40 - DNA, 54 bp, synthetic construct; identical to SEQ ID NO: 32
  source 1..54: mol_type = other DNA

SEQ ID NO: 41 - DNA, 57 bp, synthetic construct; identical to SEQ ID NO: 33
  source 1..57: mol_type = other DNA

SEQ ID NO: 42 - DNA, 60 bp, synthetic construct; identical to SEQ ID NO: 34
  source 1..60: mol_type = other DNA

SEQ ID NO: 43 - DNA, 63 bp, synthetic construct; identical to SEQ ID NO: 35
  source 1..63: mol_type = other DNA

SEQ ID NO: 44 - DNA, 39 bp, synthetic construct
  source 1..39: mol_type = other DNA
tttccgccccccgtcctagctacttccaccacctcccca

SEQ ID NO: 45 - DNA, 42 bp, synthetic construct
  source 1..42: mol_type = other DNA
tttccgccccccgtcctaactacttccaccacctcctttttc

SEQ ID NO: 46 - DNA, 70 bp, synthetic construct
  source 1..70: mol_type = other DNA
cacgacgctcttccgatctgtgctgcgcgtttcactatagggttaactttaagaaggagatatacatatg

SEQ ID NO: 47 - DNA, 70 bp, synthetic construct
  source 1..70: mol_type = other DNA
cacgacgctcttccgatctgcagctgaggaatcactatagggttaactttaagaaggagatatacatatg

SEQ ID NO: 48 - DNA, 38 bp, synthetic construct
  source 1..38: mol_type = other DNA
agacgtgtgctcttccgatcttcccgccccccgtccta

SEQ ID NO: 49 - DNA, 62 bp, synthetic construct
  source 1..62: mol_type = other DNA
aatgatacggcgaccaccgagatctacacacactctttccctacacgacgctcttccgatct

SEQ ID NO: 50 - DNA, 58 bp, synthetic construct
  source 1..58: mol_type = other DNA
caagcagaagacggcatacgagatgtgactggagttcagacgtgtgctcttccgatct

SEQ ID NO: 51 - DNA, 109 bp, synthetic construct
  source 1..109: mol_type = other DNA
ctagtaatacgactcactatagggttaactttaagaaggagatatacatatgagtcatcctcaatttgaaaaaggaggtggtggaagtagttaggacggggggcggaaa

SEQ ID NO: 52 - protein, 14 aa, synthetic construct
WSHPQFEKGGGGSS

SEQ ID NO: 53 - RNA, 77 nt, synthetic construct
  source 1..77: mol_type = other RNA
gggtgattggcgcagcctggtagcgcacttcgctggcagcgaaggggtcaggggttcgaatcccctatcacccgcca

SEQ ID NO: 54 - RNA, 77 nt, synthetic construct; identical to SEQ ID NO: 31
  source 1..77: mol_type = other RNA

SEQ ID NO: 55 - RNA, 77 nt, synthetic construct
  source 1..77: mol_type = other RNA
gggtgattggcgcagcctggtagcgcacttcgctccaaacgaaggggtcaggggttcgaatcccctatcacccgcca

SEQ ID NO: 56 - RNA, 77 nt, synthetic construct
  source 1..77: mol_type = other RNA
gggtgattggcgcagcctggtagcgcacttcgctgcggacgaaggggtcaggggttcgaatcccctatcacccgcca

SEQ ID NO: 57 - RNA, 77 nt, synthetic construct
  source 1..77: mol_type = other RNA
gggtgattggcgcagcctggtagcgcacttcgctgaaaacgaaggggtcaggggttcgaatcccctatcacccgcca

SEQ ID NO: 58 - RNA, 77 nt, synthetic construct
  source 1..77: mol_type = other RNA
gggtgattggcgcagcctggtagcgcacttcgctgataacgaaggggtcaggggttcgaatcccctatcacccgcca

SEQ ID NO: 59 - RNA, 77 nt, synthetic construct
  source 1..77: mol_type = other RNA
gggtgattggcgcagcctggtagcgcacttcgttggtaacgaaggggtcaggggttcgaatcccctatcacccgcca

SEQ ID NO: 60 - DNA, 16 bp, synthetic construct
  source 1..16: mol_type = other DNA
ctcccgccccccgtcc